European Patent Application EP 4 748 446 A2, published May 27, 2026. Title: ANTIBODY NEUTRALIZING HUMAN RESPIRATORY SYNCYTIAL VIRUS. Applicant: Merck Sharp & Dohme LLC. Application US. The sequence listing filed with the application follows.

SEQUENCE LISTING (26 sequences)

SEQ ID NO: 1 - protein, 5 aa, Homo sapiens
DSAMS

SEQ ID NO: 2 - protein, 19 aa, Homo sapiens
FIKSKTYGGTKEYAASVKG

SEQ ID NO: 3 - protein, 16 aa, Homo sapiens
GAPYGGNSDYYYGLDV

SEQ ID NO: 4 - protein, 11 aa, Homo sapiens
RTSQDVRGALA

SEQ ID NO: 5 - protein, 7 aa, Homo sapiens
DASSLET

SEQ ID NO: 6 - protein, 9 aa, Homo sapiens
QQFLDFPFT

SEQ ID NO: 7 - protein, 127 aa, synthetic construct
  REGION 1..127: note = RB-1 heavy chain with amino acid substitution
EVQLVESGGGLVRPGRSLRLSCTVSGFSFDDSAMSWVRQAPGKGLEWISFIKSKTYGGTKEYAASVKGRFTISRDDSKNIAYLQMNSLKTEDTAVYYCTRGAPYGGNSDYYYGLDVWGQGTTVTVSS

SEQ ID NO: 8 - protein, 109 aa, Homo sapiens
DIQMTQSPSSLSASVGDRVTITCRTSQDVRGALAWYQQKPGKAPKLLIFDASSLETGVPSRFSGSGSGTVFTLTISSLQPEDFAAYYCQQFLDFPFTFGQGTRLEIKRT

SEQ ID NO: 9 - protein, 127 aa, Homo sapiens
EVQLVESGGGLVRPGRSLRLSCTVSGFSFDDSAMSWVRQAPGKGLEWISFIKSKTYGGTKEYAASVKGRFTISRDDSKNIAYLQMNSLKTEDTAVYYCTRGAPYGGNSDYYYGLDVWGQGTTVIVSS

SEQ ID NO: 10 - protein, 19 aa, synthetic construct
  REGION 1..19: note = Leader sequence
MGWSCIILFLVATATGVHS

SEQ ID NO: 11 - protein, 146 aa, synthetic construct
  REGION 1..146: note = RBI VH amino acid substituted with leader
MGWSCIILFLVATATGVHSEVQLVESGGGLVRPGRSLRLSCTVSGFSFDDSAMSWVRQAPGKGLEWISFIKSKTYGGTKEYAASVKGRFTISRDDSKNIAYLQMNSLKTEDTAVYYCTRGAPYGGNSDYYYGLDVWGQGTTVTVSS

SEQ ID NO: 12 - protein, 128 aa, synthetic construct
  REGION 1..128: note = RB-1 VL and leader
MGWSCIILFLVATATGVHSDIQMTQSPSSLSASVGDRVTITCRTSQDVRGALAWYQQKPGKAPKLLIFDASSLETGVPSRFSGSGSGTVFTLTISSLQPEDFAAYYCQQFLDFPFTFGQGTRLEIKRT

SEQ ID NO: 13 - protein, 330 aa, Homo sapiens [sequence omitted]

SEQ ID NO: 14 - protein, 105 aa, Homo sapiens [sequence omitted]

SEQ ID NO: 15 - DNA, 381 bp, synthetic construct
  misc_feature 1..381: note = RB-1 with amino acid substitution
  source 1..381: mol_type = other DNA
gaggtgcagctggtggagtctgggggaggcttggtacggccagggcggtccctgagactctcctgcacagtttctggattcagctttgacgactctgctatgagctgggtccgccaggctccagggaaggggctggaatggataagtttcattaaaagtaaaacttatggtgggacaaaagaatacgccgcgtctgtgaaaggcaggttcaccatctcaagagatgattccaaaaacatcgcctatctgcaaatgaacagcctgaaaaccgaggacacagccgtgtattattgtactagaggggcgccttacggcggtaactccgattactactacggtttggacgtctggggccaagggaccacggtcactgtctcctca

SEQ ID NO: 16 - DNA, 327 bp, Homo sapiens
  source 1..327: mol_type = other DNA
gacatccagatgacccagtctccatcctccctgtctgcatctgtaggagacagagtcaccatcacttgccggacaagtcaggacgttagaggtgctttagcctggtatcaacagaaaccagggaaagctcctaaactcctgatctttgatgcctccagtttggagactggggtcccatcaaggttcagcggcagtggatctgggacagttttcactctcaccatcagcagcctgcagcctgaagattttgcagcttattactgtcagcagtttcttgatttccctttcaccttcggccaggggacacgactggaaatcaaacgtacg

SEQ ID NO: 17 - DNA, 381 bp, synthetic construct
  misc_feature 1..381: note = RB-1 VH codon optimized
  source 1..381: mol_type = other DNA
gaggtgcagctggtcgagagcgggggggggctggtgcggcctggcaggtctctgagactgagctgcaccgtgagcggcttctcctttgacgattctgccatgagctgggtgcggcaggctccaggcaagggactggagtggatctccttcatcaagtctaagacctacggcggcacaaaggagtacgccgcttccgtgaagggccggtttaccatcagcagggacgattccaagaacatcgcctatctgcagatgaacagcctgaagaccgaggacacagccgtgtactattgcacaagaggagctccttacggaggcaacagcgactactattacggactggacgtgtggggacagggaaccacagtgaccgtgagctcc

SEQ ID NO: 18 - DNA, 327 bp, synthetic construct
  misc_feature 1..327: note = RB-1 VL codon optimized
  source 1..327: mol_type = other DNA
gacattcagatgactcagtccccttcaagtctgagcgcctccgtgggcgacagagtgaccatcacatgccggaccagccaggatgtgcggggcgccctggcttggtaccagcagaagccaggcaaggcccccaagctgctgatctttgacgctagctccctggagaccggcgtgccctccaggttttctggcagcggctccggcacagtgttcaccctgacaatctctagcctgcagcctgaggactttgccgcttactattgccagcagttcctggatttccccttcaccttcggccaaggcacacggctggagatcaagaggacc

SEQ ID NO: 19 - DNA, 57 bp, synthetic construct
  misc_feature 1..57: note = Leader sequence heavy chain
  source 1..57: mol_type = other DNA
atgggttggtcctgtattatcctgttcctggtcgccactgctactggggtccactca

SEQ ID NO: 20 - DNA, 57 bp, synthetic construct
  misc_feature 1..57: note = Leader sequence light chain
  source 1..57: mol_type = other DNA
atgggctggtcctgtattatcctgttcctggtggcaaccgcaactggtgtgcatagc

SEQ ID NO: 21 - DNA, 990 bp, Homo sapiens
  source 1..990: mol_type = other DNA
gcctctacaaagggccctagcgtgttcccactggctccctcttccaagtctaccagcggaggaacagccgctctgggatgtctggtgaaggattacttcccagagcccgtgaccgtgtcctggaactctggcgccctgaccagcggagtgcacacatttccagctgtgctgcagtcctctggcctgtattccctgagctccgtggtgaccgtgccctctagctccctgggcacccagacatacatctgtaacgtgaatcacaagccaagcaatacaaaggtggacaagaaggtcgagcccaagtcctgtgataagacccacacatgccccccttgtcctgctccagagctgctgggaggacctagcgtgttcctgtttccacccaagcctaaggacaccctgatgatctctaggacccccgaggtgacatgcgtggtggtggacgtgagccacgaggatcctgaggtgaagtttaactggtacgtcgatggcgtggaggtgcacaatgccaagacaaagcccagagaggagcagtataactccacctaccgggtggtgtctgtgctgacagtgctgcaccaggactggctgaacggcaaggagtacaagtgcaaggtgtccaataaggccctgcccgctcctatcgagaagaccatctctaaggccaagggccagcctagggagccacaggtgtatacactgcctccatccagagacgagctgaccaagaaccaggtgtctctgacatgtctggtgaagggcttctacccttctgatatcgccgtggagtgggagagcaatggccagccagagaacaattataagaccacaccccctgtgctggacagcgatggctccttctttctgtacagcaagctgaccgtggataagtcccggtggcagcagggcaacgtgttcagctgttctgtgatgcacgaagccctgcacaatcactacactcagaagagcctgtccctgtcacctggtaaa

SEQ ID NO: 22 - DNA, 315 bp, Homo sapiens
  source 1..315: mol_type = other DNA
gtggccgctccctccgtgtttatcttccccccttctgacgagcagctgaagtctggcacagctagcgtggtgtgcctgctgaacaatttctaccctcgggaggccaaggtgcagtggaaggtggataacgctctgcagtctggcaatagccaggagtccgtgaccgagcaggactctaaggatagcacatattccctgtcctctaccctgacactgtctaaggccgattacgagaagcacaaggtgtatgcttgtgaagtcacccaccaggggctgagttcaccagtcaccaagtcattcaatcggggcgagtgc

SEQ ID NO: 23 - protein, 457 aa, synthetic construct
  REGION 1..457: note = RB1+YTE HEAVY CHAIN
EVQLVESGGGLVRPGRSLRLSCTVSGFSFDDSAMSWVRQAPGKGLEWISFIKSKTYGGTKEYAASVKGRFTISRDDSKNIAYLQMNSLKTEDTAVYYCTRGAPYGGNSDYYYGLDVWGQGTTVTVSSASTKGPSVFPLAPSSKSTSGGTAALGCLVKDYFPEPVTVSWNSGALTSGVHTFPAVLQSSGLYSLSSVVTVPSSSLGTQTYICNVNHKPSNTKVDKKVEPKSCDKTHTCPPCPAPELLGGPSVFLFPPKPKDTLYITREPEVTCVVVDVSHEDPEVKFNWYVDGVEVHNAKTKPREEQYNSTYRVVSVLTVLHQDWLNGKEYKCKVSNKALPAPIEKTISKAKGQPREPQVYTLPPSRDELTKNQVSLTCLVKGFYPSDIAVEWESNGQPENNYKTTPPVLDSDGSFFLYSKLTVDKSRWQQGNVFSCSVMHEALHNHYTQKSLSLSPGK

SEQ ID NO: 24 - DNA, 1374 bp, synthetic construct
  misc_feature 1..1374: note = NUCLEIC ACID ENCODING RB1+YTE HEAVY CHAIN (CODON OPTIMIZED)
  source 1..1374: mol_type = other DNA
gaggtgcagctggtggaatccggcggcggactggtcagacctggcagatccctgaggctcagctgtaccgtgagcggcttcagcttcgacgactccgccatgagctgggtgagacaggcccctggcaagggcctggagtggatcagcttcatcaagagcaaaacctatggcggaaccaaggaatacgccgcctccgtgaagggcaggttcaccatttccagggacgacagcaagaacatcgcttacctccagatgaactccctcaagaccgaggataccgccgtgtattattgcaccagaggcgccccctacggcggcaattccgactattactacggcctggatgtctggggccaaggcacaacagtgaccgtgagctccgctagcaccaagggacccagcgtgttccccctggcccccagcagcaagagcacaagcggaggaacagccgccctcggctgtctggtgaaagactacttccccgagcctgtgacagtcagctggaatagcggcgctctgaccagcggcgtccacacctttcccgctgtcctgcagagctccggcctgtacagcctgtcctccgtggtcacagtgccctcctccagcctgggcacacaaacctacatctgtaacgtgaaccacaagcccagcaacaccaaggtggacaagaaggtcgaacccaaatcctgtgacaagacccacacatgccccccctgccccgcccctgagctgctgggcggcccttccgtgttcctgttccctcccaagcccaaggataccctgtatatcaccagagaacccgaggtgacctgtgtggtggtcgacgtcagccacgaagatcctgaggtcaagttcaactggtatgtggacggcgtggaggtgcataacgccaaaaccaagcccagggaggaacagtataacagcacctacagggtggtgtccgtcctgaccgtgctgcaccaggactggctgaacggaaaggagtacaaatgtaaggtcagcaacaaagccctgcccgctcctatcgaaaagaccatctccaaggccaaaggccagcccagagaaccccaggtgtacaccctgccccctagcagagacgagctgaccaaaaaccaggtctccctgacctgcctggtgaaaggcttctaccccagcgatatcgccgtggaatgggaaagcaacggccagcctgagaacaactacaagaccacccctcccgtgctcgacagcgatggcagcttctttctgtacagcaagctgaccgtggacaagagcaggtggcaacaaggcaacgtgttctcctgctccgtgatgcacgaggctctgcacaaccactatacccagaagtccctgagcctcagccccggaaaatga

SEQ ID NO: 25 - protein, 214 aa, synthetic construct
  REGION 1..214: note = RB1+YTE LIGHT CHAIN
DIQMTQSPSSLSASVGDRVTITCRTSQDVRGALAWYQQKPGKAPKLLIFDASSLETGVPSRFSGSGSGTVFTLTISSLQPEDFAAYYCQQFLDFPFTFGQGTRLEIKRTVAAPSVFIFPPSDEQLKSGTASVVCLLNNFYPREAKVQWKVDNALQSGNSQESVTEQDSKDSTYSLSSTLTLSKADYEKHKVYACEVTHQGLSSPVTKSFNRGEC

SEQ ID NO: 26 - DNA, 642 bp, synthetic construct
  misc_feature 1..642: note = NUCLEIC ACID ENCODING RB1+YTE LIGHT CHAIN
  source 1..642: mol_type = other DNA
gacattcagatgactcagtccccttcaagtctgagcgcctccgtgggcgacagagtgaccatcacatgccggaccagccaggatgtgcggggcgccctggcttggtaccagcagaagccaggcaaggcccccaagctgctgatctttgacgctagctccctggagaccggcgtgccctccaggttttctggcagcggctccggcacagtgttcaccctgacaatctctagcctgcagcctgaggactttgccgcttactattgccagcagttcctggatttccccttcaccttcggccaaggcacacggctggagatcaagaggaccgtggccgctccctccgtgtttatcttccccccttctgacgagcagctgaagtctggcacagctagcgtggtgtgcctgctgaacaatttctaccctcgggaggccaaggtgcagtggaaggtggataacgctctgcagtctggcaatagccaggagtccgtgaccgagcaggactctaaggatagcacatattccctgtcctctaccctgacactgtctaaggccgattacgagaagcacaaggtgtatgcttgtgaagtcacccaccaggggctgagttcaccagtcaccaagtcattcaatcggggcgagtgc